European Patent Specification EP 4 021 932 B1, published October 22, 2025. Title: TCR constructs specific for EBV-derived antigens. Applicant: Max-Delbrueck-Centrum fuer Molekulare Medizin. The sequence listing filed with the application follows.

SEQUENCE LISTING (199 sequences)

SEQ ID NO: 1 - protein, 9 aa, Homo sapiens
  Epitope from LMP2A presented on A*02:01
CLGGLLTMV

SEQ ID NO: 2 - protein, 9 aa, Homo sapiens
  Epitope from LMP1 presented on B*57:01
IALYLQQNW

SEQ ID NO: 3 - protein, 9 aa, Homo sapiens
  Epitope from LMP1 presented on C*15:02
QQNWWTLLV

SEQ ID NO: 4 - protein, 9 aa, Homo sapiens
  Epitope from EBNA3C presented on C*06:02
FRKAQIQGL

SEQ ID NO: 5 - protein, 10 aa, Homo sapiens
  Epitope from EBNA3C presented on B*44:02
AEGGVGWRHW

SEQ ID NO: 6 - protein, 10 aa, Homo sapiens
  Epitope from EBNA3C presented on B*07:02
QPRAPIRPIP

SEQ ID NO: 7 - protein, 11 aa, Homo sapiens
  Epitope from EBNA3C presented on B*07:02
QPRAPIRPIPT

SEQ ID NO: 8-10 - skipped (3 entries)

SEQ ID NO: 11 - protein, 6 aa, Homo sapiens
  TCR06 - TRA - CDR1
DSAIYN

SEQ ID NO: 12 - protein, 7 aa, Homo sapiens
  TCR06 - TRA - CDR2
IQSSQRE

SEQ ID NO: 13 - protein, 11 aa, Homo sapiens
  TCR06 - TRA- CDR3
AVLMDSNYQLI

SEQ ID NO: 14 - protein, 13 aa, Homo sapiens
  TCR06 - TRA- junction aa
CAVLMDSNYQLIW

SEQ ID NO: 15 - protein, 113 aa, Homo sapiens
  TCR06 - TRA - variable region
KQEVTQIPAALSVPEGENLVLNCSFTDSAIYNLQWFRQDPGKGLTSLLLIQSSQREQTSGRLNASLDKSSGRSTLYIAASQPGDSATYLCAVLMDSNYQLIWGAGTKLIIKPD

SEQ ID NO: 16 - protein, 5 aa, Homo sapiens
  TCR06 - TRB - CDR1
WSHSY

SEQ ID NO: 17 - protein, 6 aa, Homo sapiens
  TCR06 - TRB - CDR2
SAAADI

SEQ ID NO: 18 - protein, 12 aa, Homo sapiens
  TCR06 - TRB - CDR3
ASSEDGMNTEAF

SEQ ID NO: 19 - protein, 14 aa, Homo sapiens
  TCR06 - TRB - junction aa
CASSEDGMNTEAFF

SEQ ID NO: 20 - protein, 113 aa, Homo sapiens
  TCR06 - TRB - variable region
DAGITQSPRYKITETGRQVTLMCHQTWSHSYMFWYRQDLGHGLRLIYYSAAADITDKGEVPDGYVVSRSKTENFPLTLESATRSQTSVYFCASSEDGMNTEAFFGQGTRLTVV

SEQ ID NO: 21 - protein, 6 aa, Homo sapiens
  TCR50 - TRA - CDR1
SSYSPS

SEQ ID NO: 22 - protein, 8 aa, Homo sapiens
  TCR50 - TRA - CDR2
YTSAATLV

SEQ ID NO: 23 - protein, 11 aa, Homo sapiens
  TCR50 - TRA - CDR3
VVMATGFQKLV

SEQ ID NO: 24 - protein, 13 aa, Homo sapiens
  TCR50 - TRA - junction aa
CVVMATGFQKLVF

SEQ ID NO: 25 - protein, 114 aa, Homo sapiens
  TCR50 - TRA - variable region
AQSVTQLDSHVSVSEGTPVLLRCNYSSSYSPSLFWYVQHPNKGLQLLLKYTSAATLVKGINGFEAEFKKSETSFHLTKPSAHMSDAAEYFCVVMATGFQKLVFGTGTRLLVSPN

SEQ ID NO: 26 - protein, 5 aa, Homo sapiens
  TCR50 - TRB - CDR1
SGDLS

SEQ ID NO: 27 - protein, 6 aa, Homo sapiens
  TCR50 - TRB - CDR2
YYNGEE

SEQ ID NO: 28 - protein, 12 aa, Homo sapiens
  TCR50 - TRB - CDR3
ASSVTSGSDEQF

SEQ ID NO: 29 - protein, 14 aa, Homo sapiens
  TCR50 - TRB - junction aa
CASSVTSGSDEQFF

SEQ ID NO: 30 - protein, 113 aa, Homo sapiens
  TCR50 - TRB - variable region
DSGVTQTPKHLITATGQRVTLRCSPRSGDLSVYWYQQSLDQGLQFLIQYYNGEERAKGNILERFSAQQFPDLHSELNLSSLELGDSALYFCASSVTSGSDEQFFGPGTRLTVL

SEQ ID NO: 31 - protein, 6 aa, Homo sapiens
  TCR83 - TRA - CDR1
TSGFNG

SEQ ID NO: 32 - protein, 6 aa, Homo sapiens
  TCR83 - TRA - CDR2
NVLDGL

SEQ ID NO: 33 - protein, 11 aa, Homo sapiens
  TCR83 - TRA - CDR3
AAVNNAGNMLT

SEQ ID NO: 34 - protein, 13 aa, Homo sapiens
  TCR83 - TRA - junction aa
CAAVNNAGNMLTF

SEQ ID NO: 35 - protein, 111 aa, Homo sapiens
  TCR83 - TRA - variable region
GQNIDQPTEMTATEGAIVQINCTYQTSGFNGLFWYQQHAGEAPTFLSYNVLDGLEEKGRFSSFLSRSKGYSYLLLKELQMKDSASYLCAAVNNAGNMLTFGGGTRLMVKPH

SEQ ID NO: 36 - protein, 5 aa, Homo sapiens
  TCR83 - TRB - CDR1
LGHDT

SEQ ID NO: 37 - protein, 6 aa, Homo sapiens
  TCR83 - TRB - CDR2
YNNKEL

SEQ ID NO: 38 - protein, 15 aa, Homo sapiens
  TCR83 - TRB - CDR3
ASSQGYGGPSTDTQY

SEQ ID NO: 39 - protein, 17 aa, Homo sapiens
  TCR83 - TRB - junction aa
CASSQGYGGPSTDTQYF

SEQ ID NO: 40 - protein, 116 aa, Homo sapiens
  TCR83 - TRB - variable region
DTAVSQTPKYLVTQMGNDKSIKCEQNLGHDTMYWYKQDSKKFLKIMFSYNNKELIINETVPNRFSPKSPDKAHLNLHINSLELGDSAVYFCASSQGYGGPSTDTQYFGPGTRLTVL

SEQ ID NO: 41 - protein, 5 aa, Homo sapiens
  TCR64 - TRA - CDR1
SVFSS

SEQ ID NO: 42 - protein, 7 aa, Homo sapiens
  TCR64 - TRA - CDR2
VVTGGEV

SEQ ID NO: 43 - protein, 13 aa, Homo sapiens
  TCR64 - TRA - CDR3
AGDVDTGTASKLT

SEQ ID NO: 44 - protein, 15 aa, Homo sapiens
  TCR64 - TRA - junction aa
CAGDVDTGTASKLTF

SEQ ID NO: 45 - protein, 114 aa, Homo sapiens
  TCR64 - TRA - variable region
TQLLEQSPQFLSIQEGENLTVYCNSSSVFSSLQWYRQEPGEGPVLLVTVVTGGEVKKLKRLTFQFGDARKDSSLHITAAQPGDTGLYLCAGDVDTGTASKLTFGTGTRLQVTLD

SEQ ID NO: 46 - protein, 5 aa, Homo sapiens
  TCR64 - TRB - CDR1
MDHEN

SEQ ID NO: 47 - protein, 6 aa, Homo sapiens
  TCR64 - TRB - CDR2
SYDVKM

SEQ ID NO: 48 - protein, 14 aa, Homo sapiens
  TCR64 - TRB - CDR3
ASSLLGSGALYEQY

SEQ ID NO: 49 - protein, 16 aa, Homo sapiens
  TCR64 - TRB - junction aa
CASSLLGSGALYEQYF

SEQ ID NO: 50 - protein, 115 aa, Homo sapiens
  TCR64 - TRB - variable region
DVKVTQSSRYLVKRTGEKVFLECVQDMDHENMFWYRQDPGLGLRLIYFSYDVKMKEKGDIPEGYSVSREKKERFSLILESASTNQTSMYLCASSLLGSGALYEQYFGPGTRLTVT

SEQ ID NO: 51 - protein, 6 aa, Homo sapiens
  CDR25 - TRA - CDR1
SSYSPS

SEQ ID NO: 52 - protein, 8 aa, Homo sapiens
  CDR25 - TRA - CDR2
YTSAATLV

SEQ ID NO: 53 - protein, 11 aa, Homo sapiens
  CDR25 - TRA - CDR3
VAWDTGFQKLV

SEQ ID NO: 54 - protein, 13 aa, Homo sapiens
  CDR25 - TRA - junction aa
CVAWDTGFQKLVF

SEQ ID NO: 55 - protein, 114 aa, Homo sapiens
  CD25 - TRA - variable region
AQSVTQLDSHVSVSEGTPVLLRCNYSSSYSPSLFWYVQHPNKGLQLLLKYTSAATLVKGINGFEAEFKKSETSFHLTKPSAHMSDAAEYFCVAWDTGFQKLVFGTGTRLLVSPN

SEQ ID NO: 56 - protein, 5 aa, Homo sapiens
  CD25 - TRB - CDR1
SNHLY

SEQ ID NO: 57 - protein, 6 aa, Homo sapiens
  CD25 - TRB - CDR2
FYNNEI

SEQ ID NO: 58 - protein, 10 aa, Homo sapiens
  CD25 - TRB - CDR3
ASKALADTQY

SEQ ID NO: 59 - protein, 12 aa, Homo sapiens
  CD25 - TRB - junction aa
CASKALADTQYF

SEQ ID NO: 60 - protein, 112 aa, Homo sapiens
  TCR25 - TRB - variable region
EPEVTQTPSHQVTQMGQEVILRCVPISNHLYFYWYRQILGQKVEFLVSFYNNEISEKSEIFDDQFSVERPDGSNFTLKIRSTKLEDSAMYFCASKALADTQYFGPGTRLTVL

SEQ ID NO: 61 - protein, 6 aa, Homo sapiens
  TCR58 - TRA - CDR1
NSASQS

SEQ ID NO: 62 - protein, 6 aa, Homo sapiens
  TCR58 - TRA - CDR2
VYSSGN

SEQ ID NO: 63 - protein, 11 aa, Homo sapiens
  TCR58 - TRA - CDR3
VASGDSSYKLI

SEQ ID NO: 64 - protein, 13 aa, Homo sapiens
  TCR58 - TRA - junction aa
CVASGDSSYKLIF

SEQ ID NO: 65 - protein, 111 aa, Homo sapiens
  TCR58 - TRA - variable region
RKEVEQDPGPFNVPEGATVAFNCTYSNSASQSFFWYRQDCRKEPKLLMSVYSSGNEDGRFTAQLNRASQYISLLIRDSKLSDSATYLCVASGDSSYKLIFGSGTRLLVRPD

SEQ ID NO: 66 - protein, 5 aa, Homo sapiens
  TCR58 - TRB - CDR1
SNHLY

SEQ ID NO: 67 - protein, 6 aa, Homo sapiens
  TCR58 - TRB - CDR2
FYNNEI

SEQ ID NO: 68 - protein, 13 aa, Homo sapiens
  TCR58 - TRB - CDR3
ASSDPLSTYNEQF

SEQ ID NO: 69 - protein, 15 aa, Homo sapiens
  TCR58 - TRB - junction aa
CASSDPLSTYNEQFF

SEQ ID NO: 70 - protein, 115 aa, Homo sapiens
  TCR58 - TRB - variable region
EPEVTQTPSHQVTQMGQEVILRCVPISNHLYFYWYRQILGQKVEFLVSFYNNEISEKSEIFDDQFSVERPDGSNFTLKIRSTKLEDSAMYFCASSDPLSTYNEQFFGPGTRLTVL

SEQ ID NO: 71 - protein, 7 aa, Homo sapiens
  TCR27 - TRA - CDR1
TISGTDY

SEQ ID NO: 72 - protein, 5 aa, Homo sapiens
  TCR27 - TRA - CDR2
GLTSN

SEQ ID NO: 73 - protein, 14 aa, Homo sapiens
  TCR27 - TRA - CDR3
ILCGAGGTSYGKLT

SEQ ID NO: 74 - protein, 16 aa, Homo sapiens
  TCR27 - TRA - junction aa
CILCGAGGTSYGKLTF

SEQ ID NO: 75 - protein, 114 aa, Homo sapiens
  TCR27 - TRA - variable region
DAKTTQPNSMESNEEEPVHLPCNHSTISGTDYIHWYRQLPSQGPEYVIHGLTSNVNNRMASLAIAEDRKSSTLILHRATLRDAAVYYCILCGAGGTSYGKLTFGQGTILTVHPN

SEQ ID NO: 76 - protein, 5 aa, Homo sapiens
  TCR27 - TRB - CDR1
MNHEY

SEQ ID NO: 77 - protein, 6 aa, Homo sapiens
  TCR27 - TRB - CDR2
SMNVEV

SEQ ID NO: 78 - protein, 12 aa, Homo sapiens
  TCR27 - TRB - CDR3
ASNVQGANNEQF

SEQ ID NO: 79 - protein, 14 aa, Homo sapiens
  TCR27 - TRB - junction aa
CASNVQGANNEQFF

SEQ ID NO: 80 - protein, 113 aa, Homo sapiens
  TCR27 - TRB - variable region
EAQVTQNPRYLITVTGKKLTVTCSQNMNHEYMSWYRQDPGLGLRQIYYSMNVEVTDKGDVPEGYKVSRKEKRNFPLILESPSPNQTSLYFCASNVQGANNEQFFGPGTRLTVL

SEQ ID NO: 81 - protein, 7 aa, Homo sapiens
  TCR01 - TRA - CDR1
TISGTDY

SEQ ID NO: 82 - protein, 5 aa, Homo sapiens
  TCR01 - TRA - CDR2
GLTSN

SEQ ID NO: 83 - protein, 14 aa, Homo sapiens
  TCR01 - TRA - CDR3
ILCGAGGTSYGKLT

SEQ ID NO: 84 - protein, 16 aa, Homo sapiens
  TCR01 - TRA - junction aa
CILCGAGGTSYGKLTF

SEQ ID NO: 85 - protein, 114 aa, Homo sapiens; identical to SEQ ID NO: 75
  TCR01 - TRA - variable region

SEQ ID NO: 86 - protein, 5 aa, Homo sapiens
  TCR01 - TRB - CDR1
MNHEY

SEQ ID NO: 87 - protein, 6 aa, Homo sapiens
  TCR01 - TRB - CDR2
SMNVEV

SEQ ID NO: 88 - protein, 12 aa, Homo sapiens
  TCR01 - TRB - CDR3
ASAIQGANNEQF

SEQ ID NO: 89 - protein, 14 aa, Homo sapiens
  TCR01 - TRB - junction aa
CASAIQGANNEQFF

SEQ ID NO: 90 - protein, 113 aa, Homo sapiens
  TCR01 - TRB - variable region
EAQVTQNPRYLITVTGKKLTVTCSQNMNHEYMSWYRQDPGLGLRQIYYSMNVEVTDKGDVPEGYKVSRKEKRNFPLILESPSPNQTSLYFCASAIQGANNEQFFGPGTRLTVL

SEQ ID NO: 91 - DNA, 339 bp, Artificial Sequence
  DNA encoding variable region of TCR06 - TRA
aagcaagaagtgacccagattcctgccgctctgtccgtgcctgaaggcgagaatctggtcctgaactgcagcttcaccgacagcgccatctacaacctgcagtggttcaggcaggatcccggcaagggactgacaagcctgctgctgattcagagcagccagagagagcagacctccggcagactgaatgccagcctggataagtccagcggcagaagcaccctgtatatcgccgcttctcagcctggcgatagcgccacatatctgtgtgccgtcctgatggactccaactaccagctgatttggggagccggcaccaagctgatcatcaagcccgac

SEQ ID NO: 92 - DNA, 339 bp, Artificial Sequence
  DNA encoding variable region of TCR06 - TRB
gatgccggaatcacacagagccccagatacaagatcaccgagacaggccggcaagtgaccctgatgtgtcaccagacatggtcccacagctacatgttctggtacagacaggacctcggccacggcctgagactgatctactattctgccgccgctgacatcaccgacaagggcgaagtgcctgatggctacgtggtgtccagaagcaagaccgagaacttcccactgacactggaaagcgccacacggtcccagaccagcgtgtacttttgtgccagcagcgaggacggaatgaacaccgaggcctttttcggccaaggcaccagactgaccgtggtg

SEQ ID NO: 93 - DNA, 342 bp, Artificial Sequence
  DNA encoding variable region of TCR50 - TRA
gcccagagcgtgacacaactggatagccacgtgtccgtgtctgagggcacacctgtgctgctgagatgcaactactccagcagctacagccccagcctgttttggtacgtgcagcaccctaacaagggactgcagctgctgctgaagtacacctctgccgccacactggtcaagggcatcaatggcttcgaggccgagttcaagaagtccgagacaagcttccacctgaccaagcctagcgctcacatgtccgatgccgccgaatacttctgcgtggtcatggccaccggcttccagaaactggtgtttggcacaggcacccggctgctcgtgtccccaaat

SEQ ID NO: 94 - DNA, 339 bp, Artificial Sequence
  DNA encoding variable region of TCR50 - TRB
gatagcggcgttacccagacacctaagcacctgatcacagccacaggccagcgcgtgaccctgagatgttctcctagaagcggcgacctgagcgtgtactggtatcagcagtctctggaccagggcctgcagttcctgatccagtactacaacggcgaggaaagagccaagggcaacatcctggaacggttcagcgcccagcagttcccagatctgcacagcgagctgaacctgagcagcctggaactgggagatagcgccctgtacttctgtgccagctctgtgaccagcggcagcgacgagcagttttttggccctggcaccagactgaccgtgctg

SEQ ID NO: 95 - DNA, 333 bp, Artificial Sequence
  DNA encoding variable region of TCR83 - TRA
ggccagaacatcgatcagcctacagagatgaccgccaccgagggcgccatcgtgcagatcaattgcacctaccagaccagcggcttcaacggcctgttctggtatcagcagcatgccggcgaggcccctaccttcctgagctacaatgtgctggacggcctggaagaaaagggcagattcagcagcttcctgtccagaagcaagggctactcctacctgctgctgaaagaactgcagatgaaggacagcgcctcttacctgtgtgccgccgtgaacaacgccggcaacatgctgacatttggcggcggaacacggctgatggtcaagccccac

SEQ ID NO: 96 - DNA, 348 bp, Artificial Sequence
  DNA encoding variable region of TCR83 - TRB
gatacagccgtgtctcagacccctaagtacctggtcacccagatgggcaacgacaagagcatcaagtgcgagcagaacctgggccacgacaccatgtactggtacaagcaggacagcaagaaattcctgaagatcatgttcagctacaacaacaaagagctgatcatcaacgagacagtgcccaaccggttcagccctaagagccctgataaggcccacctgaacctgcacatcaacagcctggaactgggcgacagcgccgtgtacttttgtgccagctctcaaggctatggcggccctagcaccgacacacagtatttcggccctggcaccagactgaccgtgctg

SEQ ID NO: 97 - DNA, 342 bp, Artificial Sequence
  DNA encoding variable region of TCR64 - TRA
acacagctgctggaacagagcccacagttcctgagcatccaagagggcgagaacctgaccgtgtactgcaacagcagcagcgtgttcagctccctgcagtggtacaggcaagagcctggcgaaggacctgtgctgctggtcacagttgtgacaggcggcgaagtgaagaagctgaagcggctgaccttccagttcggcgacgccagaaaggattccagcctgcacattaccgctgctcagccaggcgataccggcctgtatctttgtgctggcgacgtcgacacaggcaccgccagcaaactgacatttggcaccggcaccaggctgcaagtgaccctggac

SEQ ID NO: 98 - DNA, 345 bp, Artificial Sequence
  DNA encoding variable region of TCR64 - TRB
gacgtgaaagtgacacagagcagcagatacctggtcaagcggaccggcgagaaggtgttcctggaatgcgtgcaggacatggaccacgagaatatgttctggtacagacaggaccccggcctgggcctgagactgatctacttcagctacgacgtgaagatgaaggaaaagggcgacatccccgagggctacagcgtgtccagagagaagaaagagcggttcagcctgatcctggaaagcgccagcaccaaccagaccagcatgtacctgtgtgccagcagcctgcttggatctggcgccctgtacgagcagtatttcggccctggcaccagactgaccgtgacc

SEQ ID NO: 99 - DNA, 342 bp, Artificial Sequence
  DNA encoding variable region of TCR25 - TRA
gcccagagcgtgacacaactggatagccacgtgtccgtgtctgagggcacacctgtgctgctgagatgcaactactccagcagctacagccccagcctgttttggtacgtgcagcaccctaacaagggcctgcagctgctgctgaagtacacatctgccgccacactggtcaagggcatcaatggcttcgaggccgagttcaagaagtctgagacaagcttccacctgaccaagcctagcgctcacatgtccgatgccgccgaatacttctgcgtggcctgggataccggcttccagaaactggtgtttggcaccggcacacggctgctcgtgtccccaaat

SEQ ID NO: 100 - DNA, 336 bp, Artificial Sequence
  DNA encoding variable region of TCR25 - TRB
gagcccgaagtgacacagacacccagccaccaagtgacccagatgggccaagaagtgatcctgcgctgcgtgcccatcagcaaccacctgtacttctactggtacagacagatcctgggccagaaagtcgagttcctggtgtccttctacaacaacgagatcagcgagaagtccgagatcttcgacgaccagttcagcgtggaaagacccgacggcagcaacttcaccctgaagatcagaagcaccaagctcgaggacagcgccatgtacttttgcgcctctaaggccctggccgacacacagtattttggccctggcaccagactgaccgtgctg

SEQ ID NO: 101 - DNA, 333 bp, Artificial Sequence
  DNA encoding variable region of TCR58 - TRA
cggaaagaggtggaacaggaccctggacctttcaacgttccagagggcgccaccgtggccttcaattgcacctacagcaatagcgccagccagagctttttctggtatcggcaggactgccggaaagaacccaagctgctgatgagcgtgtacagcagcggcaacgaggacggcagattcacagcccagctgaacagagccagccagtacatctccctgctgatccgggatagcaagctgagcgatagcgccacctatctgtgtgtggccagcggcgatagcagctacaagctgatctttggcagcggcaccaggctgcttgtgcggcccgat

SEQ ID NO: 102 - DNA, 345 bp, Artificial Sequence
  DNA encoding variable region of TCR58 - TRB
gagcccgaagtgacacagacacccagccaccaagtgacccagatgggccaagaagtgatcctgcgctgcgtgcccatcagcaaccacctgtacttctactggtacagacagatcctgggccagaaagtcgagttcctggtgtccttctacaacaacgagatcagcgagaagtccgagatcttcgacgaccagttcagcgtggaaagacccgacggcagcaacttcaccctgaagatcagaagcaccaagctcgaggacagcgccatgtacttttgcgccagcagcgatcccctgagcacctacaacgagcagttcttcggccctggcaccagactgaccgtgctg

SEQ ID NO: 103 - DNA, 342 bp, Artificial Sequence
  DNA encoding variable region of TCR27 - TRA
gacgccaagaccacacagcccaacagcatggaaagcaacgaagaggaacccgtgcatctgccctgcaaccacagcacaatcagcggcaccgactacatccactggtatagacagctgccctctcagggccccgagtatgtgattcacggactgaccagcaacgtgaacaaccggatggcctctctggccattgccgaggacagaaagagcagcaccctgatcctgcacagagccacactgagagatgccgccgtgtactactgcatcctttgtggcgctggcggcaccagctatggcaagctgacatttggccagggcaccatcctgaccgtgcatcccaac

SEQ ID NO: 104 - DNA, 339 bp, Artificial Sequence
  DNA encoding variable region of TCR27 - TRB
gaagctcaagtgacacagaaccccagatacctgatcaccgtgaccggcaagaaactgaccgtgacctgcagccagaacatgaaccacgagtacatgagctggtacagacaggaccctggcctgggcctgagacagatctactacagcatgaacgtggaagtgaccgacaagggcgacgtgcccgagggctacaaggtgtccagaaaagagaagcggaacttcccactgatcctggaaagcccatctcctaaccagaccagcctgtacttctgcgccagcaatgtgcagggcgccaacaacgagcagttcttcggccctggcaccagactgacagtgctg

SEQ ID NO: 105 - DNA, 342 bp, Artificial Sequence; identical to SEQ ID NO: 103
  DNA encoding variable region of TCR01 - TRA

SEQ ID NO: 106 - DNA, 339 bp, Artificial Sequence
  DNA encoding variable region of TCR01 - TRB
gaagctcaagtgacacagaaccccagatacctgatcaccgtgaccggcaagaaactgaccgtgacctgcagccagaacatgaaccacgagtacatgagctggtacagacaggaccctggcctgggcctgagacagatctactacagcatgaacgtggaagtgaccgacaagggcgacgtgcccgagggctacaaggtgtccagaaaagagaagcggaacttcccactgatcctggaaagcccatctcctaaccagaccagcctgtacttctgcgccagcgctattcagggcgccaacaacgagcagttcttcggccctggcaccagactgacagtgctg

SEQ ID NO: 107 - protein, 9 aa, Homo sapiens
WTLLVDLLW

SEQ ID NO: 108 - protein, 10 aa, Homo sapiens
IALYLQQNWW

SEQ ID NO: 109 - protein, 10 aa, Homo sapiens
WWTLLVDLLW

SEQ ID NO: 110 - protein, 10 aa, Homo sapiens
IIALYLQQNW

SEQ ID NO: 111 - protein, 10 aa, Homo sapiens
WTLLVDLLWL

SEQ ID NO: 112 - protein, 9 aa, Homo sapiens
LAILIWMYY

SEQ ID NO: 113 - protein, 9 aa, Homo sapiens
LLFLAILIW

SEQ ID NO: 114 - protein, 10 aa, Homo sapiens
LLLFLAILIW

SEQ ID NO: 115 - protein, 10 aa, Homo sapiens
LAILIWMYYH

SEQ ID NO: 116 - protein, 9 aa, Homo sapiens
ALYLQQNWW

SEQ ID NO: 117 - protein, 10 aa, Homo sapiens
FLAILIWMYY

SEQ ID NO: 118 - protein, 9 aa, Homo sapiens
NSNEGRHHL

SEQ ID NO: 119 - protein, 497 aa, Homo sapiens
  LMP2A
MGSLEMVPMGAGPPSPGGDPDGYDGGNNSQYPSASGSSGNTPTPPNDEERESNEEPPPPYEDPYWGNGDRHSDYQPLGTQDQSLYLGLQHDGNDGLPPPPYSPRDDSSQHIYEEAGRGSMNPVCLPVIVAPYLFWLAAIAASCFTASVSTVVTATGLALSLLLLAAVASSYAAAQRKLLTPVTVLTAVVTFFAICLTWRIEDPPFNSLLFALLAAAGGLQGIYVLVMLVLLILAYRRRWRRLTVCGGIMFLACVLVLIVDAVLQLSPLLGAVTVVSMTLLLLAFVLWLSSPGGLGTLGAALLTLAAALALLASLILGTLNLTTMFLLMLLWTLVVLLICSSCSSCPLSKILLARLFLYALALLLLASALIAGGSILQTNFKSLSSTEFIPNLFCMLLLIVAGILFILAILTEWGSGNRTYGPVFMCLGGLLTMVAGAVWLTVMSNTLLSAWILTAGFLIFLIGFALFGVIRCCRYCCYYCLTLESEERPPTPYRNTV

SEQ ID NO: 120 - protein, 386 aa, Homo sapiens
  LMP1
MEHDLERGPPGPRRPPRGPPLSSSLGLALLLLLLALLFWLYIVMSDWTGGALLVLYSFALMLIIIILIIFIFRRDLLCPLGALCILLLMITLLLIALWNLHGQALFLGIVLFIFGCLLVLGIWIYLLEMLWRLGATIWQLLAFFLAFFLDLILLIIALYLQQNWWTLLVDLLWLLLFLAILIWMYYHGQRHSDEHHHDDSLPHPQQATDDSGHESDSNSNEGRHHLLVSGAGDGPPLCSQNLGAPGGGPDNGPQDPDNTDDNGPQDPDNTDDNGPHDPLPQDPDNTDDNGPQDPDNTDDNGPHDPLPHSPSDSAGNDGGPPQLTEEVENKGGDQGPPLMTDGGGGHSHDSGHGGGDPHLPTLLLGSSGSGGDDDDPHGPVQLSYYD

SEQ ID NO: 121 - protein, 992 aa, Homo sapiens
  EBNA3C
MESFEGQGDSRQSPDNERGDNVQTTGEHDQDPGPGPPSSGASERLVPEESYSRDQQPWGQSRGDENRGWMQRIRRRRRRRAALSGHLLDTEDNVPPWLPPHDITPYTARNIRDAACRAVKQSHLQALSNLILDSGLDTQHILCFVMAARQRLQDIRRGPLVAEGGVGWRHWLLTSPSQSWPMGYRTATLRTLTPVPNRVGADSIMLTATFGCQNAARTLNTFSATVWTPPHAGPREQERYAREAEVRFLRGKWQRRYRRIYDLIELCGSLHHIWQNLLQTEENLLDFVRFMGVMSSCNNPAVNYWFHKTIGNFKPYYPWNAPPNENPYHARRGIKEHVIQNAFRKAQIQGLSMLATGGEPRGDATSETSSDEDTGRQGSDVELESSDDELPYIDPNMEPVQQRPVMFVSRVPAKKPRKLPWPTPKTHPVKRTNVKTSDRSDKAEAQSTPERPGPSEQSSVTVEPAHPTPVEMPMVILHQPPPVPKPVPVKPTPPPSRRRRGACVVYDDDVIEVIDVETTEDSSSVSQPNKPHRKHQDGFQRSGRRQKRAAPPTVSPSDTGPPAVGPPAAGPPAAGPPAAGPPAAGPPAAGPPAAGPRILAPLSAGPPAAGPHIVTPPSARPRIMAPPVVRMFMRERQLPQSTGRKPQCFWEMRAGREITQMQQEPSSHLQSATQPTTPRPSWAPSVCALSVMDAGKAQPIESSHLSSMSPTQPISHEEQPRYEDPDAPLDLSLHPDVAAQPAPQAPYQGYQEPPAPQAPYQGYQEPPPPQAPYQGYQEPPAHGLQSSSYPGYAGPWTPRSQHPCYRHPWAPWSQDPVHGHTQGPWDPRAPHLPPQWDGSAGHGQDQVSQFPHLQSETGPPRLQLSLVPLVSSSAPSWSSPQPRAPIRPIPTRFPPPPMPLQDSMAVGCDSSGTACPSMPFASDYSQGAFTPLDINATTPKRPRVEESSHGPARCSQATAEAQEILSDNSEISVFPKDAKQTDYDASTESELD

SEQ ID NO: 122 - protein, 14 aa, Homo sapiens
AMSDLYAGNNRKLI

SEQ ID NO: 123 - protein, 11 aa, Homo sapiens
ALTFLRDDKII

SEQ ID NO: 124 - protein, 15 aa, Homo sapiens
ASSQDARVSGANVLT

SEQ ID NO: 125 - protein, 12 aa, Homo sapiens
ASSVTSGSDEQF

SEQ ID NO: 126 - protein, 13 aa, Homo sapiens
ASSFSLGHSYEQY

SEQ ID NO: 127 - protein, 9 aa, Homo sapiens
QPRAPIRPI

SEQ ID NO: 128 - protein, 12 aa, Homo sapiens
RPIPTRFPPPPM

SEQ ID NO: 129 - protein, 12 aa, Homo sapiens
RPRVEESSHGPA

SEQ ID NO: 130 - protein, 8 aa, Homo sapiens
SPQPRAPI

SEQ ID NO: 131 - protein, 11 aa, Homo sapiens
SPQPRAPIRPI

SEQ ID NO: 132 - protein, 12 aa, Homo sapiens
SPQPRAPIRPIP

SEQ ID NO: 133 - protein, 10 aa, Homo sapiens
PQPRAPIRPI

SEQ ID NO: 134 - protein, 10 aa, Homo sapiens
QPRAPIRPIP

SEQ ID NO: 135 - protein, 8 aa, Homo sapiens
PRAPIRPI

SEQ ID NO: 136 - protein, 10 aa, Homo sapiens
APIRPIPTRF

SEQ ID NO: 137 - protein, 8 aa, Homo sapiens
FPPPPMPL

SEQ ID NO: 138 - protein, 10 aa, Homo sapiens
HGPARCSQAT

SEQ ID NO: 139 - protein, 9 aa, Homo sapiens
RPIPTRFPP

SEQ ID NO: 140 - protein, 8 aa, Homo sapiens
RPIPTRFP

SEQ ID NO: 141 - protein, 11 aa, Homo sapiens
IPTRFPPPPMP

SEQ ID NO: 142 - protein, 11 aa, Homo sapiens
PIPTRFPPPPM

SEQ ID NO: 143 - protein, 12 aa, Homo sapiens
IPTRFPPPPMPL

SEQ ID NO: 144 - protein, 10 aa, Homo sapiens
GPARCSQATA

SEQ ID NO: 145 - protein, 12 aa, Homo sapiens
FPPPPMPLQDSM

SEQ ID NO: 146 - protein, 9 aa, Homo sapiens
PPMPLQDSM

SEQ ID NO: 147 - protein, 10 aa, Homo sapiens
RPIPTRFPPP

SEQ ID NO: 148 - protein, 10 aa, Homo sapiens
MPLQDSMAVG

SEQ ID NO: 149 - protein, 12 aa, Homo sapiens
PIPTRFPPPPMP

SEQ ID NO: 150 - protein, 10 aa, Homo sapiens
PMPLQDSMAV

SEQ ID NO: 151 - protein, 8 aa, Homo sapiens
PMPLQDSM

SEQ ID NO: 152 - protein, 11 aa, Homo sapiens
QPRAPIRPIPT

SEQ ID NO: 153 - protein, 8 aa, Homo sapiens
QPRAPIRP

SEQ ID NO: 154 - protein, 9 aa, Homo sapiens
RAPIRPIPT

SEQ ID NO: 155 - protein, 10 aa, Homo sapiens
SERLVPEESY

SEQ ID NO: 156 - protein, 10 aa, Homo sapiens
WLLTSPSQSW

SEQ ID NO: 157 - protein, 9 aa, Homo sapiens
LLTSPSQSW

SEQ ID NO: 158 - protein, 9 aa, Homo sapiens
RRYRRIYDL

SEQ ID NO: 159 - protein, 9 aa, Homo sapiens
AREAEVRFL

SEQ ID NO: 160 - protein, 9 aa, Homo sapiens
LRGKWQRRY

SEQ ID NO: 161 - protein, 9 aa, Homo sapiens
ERYAREAEV

SEQ ID NO: 162 - protein, 9 aa, Homo sapiens
SRRRRGACV

SEQ ID NO: 163 - protein, 9 aa, Homo sapiens
NLLDFVRFM

SEQ ID NO: 164 - protein, 9 aa, Homo sapiens
RRIYDLIEL

SEQ ID NO: 165 - protein, 9 aa, Homo sapiens
RRRRGACVV

SEQ ID NO: 166 - protein, 9 aa, Homo sapiens
VRFLRGKWQ

SEQ ID NO: 167 - protein, 9 aa, Homo sapiens
RRRGACVVY

SEQ ID NO: 168 - protein, 9 aa, Homo sapiens
QRRYRRIYD

SEQ ID NO: 169 - protein, 9 aa, Homo sapiens
VRFMGVMSS

SEQ ID NO: 170 - protein, 10 aa, Homo sapiens
YAREAEVRFL

SEQ ID NO: 171 - protein, 9 aa, Homo sapiens
NRVGADSIM

SEQ ID NO: 172 - protein, 9 aa, Homo sapiens
LHHIWQNLL

SEQ ID NO: 173 - protein, 9 aa, Homo sapiens
RRGIKEHVI

SEQ ID NO: 174 - protein, 9 aa, Homo sapiens
YRRIYDLIE

SEQ ID NO: 175 - protein, 10 aa, Homo sapiens
RRYRRIYDLI

SEQ ID NO: 176 - protein, 9 aa, Homo sapiens
ARRGIKEHV

SEQ ID NO: 177 - protein, 10 aa, Homo sapiens
QRRYRRIYDL

SEQ ID NO: 178 - protein, 9 aa, Homo sapiens
WQRRYRRIY

SEQ ID NO: 179 - protein, 10 aa, Homo sapiens
FLRGKWQRRY

SEQ ID NO: 180 - protein, 9 aa, Homo sapiens
RRGACVVYD

SEQ ID NO: 181 - protein, 9 aa, Homo sapiens
VYDDDVIEV

SEQ ID NO: 182 - protein, 9 aa, Homo sapiens
YAREAEVRF

SEQ ID NO: 183 - protein, 9 aa, Homo sapiens
GCQNAARTL

SEQ ID NO: 184 - protein, 9 aa, Homo sapiens
NSNEGRHHL

SEQ ID NO: 185 - protein, 9 aa, Homo sapiens
DSLPHPQQA

SEQ ID NO: 186 - protein, 9 aa, Homo sapiens
YLQQNWWTL

SEQ ID NO: 187 - protein, 10 aa, Homo sapiens
FMCLGGLLTM

SEQ ID NO: 188 - protein, 9 aa, Homo sapiens
MLLLIVAGI

SEQ ID NO: 189 - protein, 9 aa, Homo sapiens
NLFCMLLLI

SEQ ID NO: 190 - protein, 10 aa, Homo sapiens
LLIVAGILFI

SEQ ID NO: 191 - protein, 10 aa, Homo sapiens
NLFCMLLLIV

SEQ ID NO: 192 - protein, 10 aa, Homo sapiens
MCLGGLLTMV

SEQ ID NO: 193 - protein, 9 aa, Homo sapiens
LIVAGILFI

SEQ ID NO: 194 - protein, 9 aa, Homo sapiens
FIPNLFCML

SEQ ID NO: 195 - protein, 9 aa, Homo sapiens
IVAGILFIL

SEQ ID NO: 196 - protein, 10 aa, Homo sapiens
MLLLIVAGIL

SEQ ID NO: 197 - protein, 10 aa, Homo sapiens
CMLLLIVAGI

SEQ ID NO: 198 - protein, 10 aa, Homo sapiens
PNLFCMLLLI

SEQ ID NO: 199 - protein, 10 aa, Homo sapiens
FIPNLFCMLL